European Patent Application EP 4 624 492 A1, published October 1, 2025. Title: Anti-CCR8 Antibodies and Uses Thereof. Applicant: SHANGHAI HONGCHENG BIOPHARMACEUTICAL CO., LTD. Application US. The sequence listing filed with the application follows.

SEQUENCE LISTING (95 sequences)

SEQ ID NO: 1 - protein, 5 aa, artificial sequence
AYAMN

SEQ ID NO: 2 - protein, 19 aa, artificial sequence
RIRSKSNNFATYYADSVTD

SEQ ID NO: 3 - protein, 12 aa, artificial sequence
HGRRDLLYSMDF

SEQ ID NO: 4 - protein, 5 aa, artificial sequence
DYYVN

SEQ ID NO: 5 - protein, 17 aa, artificial sequence
VINPHNGDTRYNQKFKG

SEQ ID NO: 6 - protein, 10 aa, artificial sequence
WLRRGYYFDS

SEQ ID NO: 7 - protein, 5 aa, artificial sequence
GYNMN

SEQ ID NO: 8 - protein, 17 aa, artificial sequence
NIDPYYGGTNYNQKFKG

SEQ ID NO: 9 - protein, 18 aa, artificial sequence
ETWFITTGVIKKGFYFDY

SEQ ID NO: 10 - protein, 19 aa, artificial sequence
RIRSKSNDFATYYADSVKG

SEQ ID NO: 11 - protein, 19 aa, artificial sequence
RIRSKSNNFATYYADSVKD

SEQ ID NO: 12 - protein, 16 aa, artificial sequence
RSSKSLLHSNGITYLF

SEQ ID NO: 13 - protein, 7 aa, artificial sequence
QMSNLAS

SEQ ID NO: 14 - protein, 8 aa, artificial sequence
AQSLELPL

SEQ ID NO: 15 - protein, 11 aa, artificial sequence
RASQSISDYLH

SEQ ID NO: 16 - protein, 7 aa, artificial sequence
YVSQSIS

SEQ ID NO: 17 - protein, 9 aa, artificial sequence
QNGHSFPLT

SEQ ID NO: 18 - protein, 12 aa, artificial sequence
SASSIISSNYLH

SEQ ID NO: 19 - protein, 7 aa, artificial sequence
RTSSLAS

SEQ ID NO: 20 - protein, 9 aa, artificial sequence
QQGSSIPRT

SEQ ID NO: 21 - protein, 123 aa, artificial sequence
EVQLVESGGGLVQPGGSLKLSCAASGFNFNAYAMNWVRQASGKGLEWVGRIRSKSNNFATYYADSVTDRFTISRDDSKNTAYLQMNSLKTEDTAVYYCVRHGRRDLLYSMDFWGQGTTVTVSS

SEQ ID NO: 22 - protein, 123 aa, artificial sequence
EVQLVESGGGLVQPGGSLKLSCAASGFTFSAYAMNWVRQASGKGLEWVGRIRSKSNNFATYYADSVTDRFTISRDDSKNTAYLQMNSLKTEDTAVYYCVRHGRRDLLYSMDFWGQGTTVTVSS

SEQ ID NO: 23 - protein, 123 aa, artificial sequence
EVQLVESGGGLVQPGGSLKLSCAASGFTFSAYAMNWVRQASGKGLEWVARIRSKSNNFATYYADSVTDRFTISRDDSKSTLYLQMNSLKTEDTAVYYCVRHGRRDLLYSMDFWGQGTTVTVSS

SEQ ID NO: 24 - protein, 123 aa, artificial sequence
EVQLVESGGGLVQPGGSLKLSCAASGFNFNAYAMNWVRQASGKGLEWVARIRSKSNNFATYYADSVTDRFTISRDDSKSTLYLQMNSLKTEDTAVYYCVRHGRRDLLYSMDFWGQGTTVTVSS

SEQ ID NO: 25 - protein, 123 aa, artificial sequence
EVQLVESGGGLVQPGGSLKLSCAASGFNFNAYAMNWVRQASGKGLEWVARIRSKSNDFATYYADSVKDRFTISRDDSKSTLYLQMNSLKTEDTAVYYCVRHGRRDLLYSMDFWGQGTTVTVSS

SEQ ID NO: 26 - protein, 123 aa, artificial sequence
EVQLVESGGGLVQPGGSLKLSCAASGFNFNAYAMNWVRQASGKGLEWVARIRSKSNDFATYYADSVKGRFTISRDDSKNTLYLQMNSLKTEDTAVYYCVRHGRRDLLYSMDFWGQGTTVTVSS

SEQ ID NO: 27 - protein, 123 aa, artificial sequence
EVQLVESGGGLVQPGGSLKLSCAASGFNFNAYAMNWVRQASGKGLEWVARIRSKSNNFATYYADSVKDRFTISRDDSKSTVYLQMNSLKTEDTAVYYCVRHGRRDLLYSMDFWGQGTTVTVSS

SEQ ID NO: 28 - protein, 119 aa, artificial sequence
QVQLVQSGAEVKKPGASVKVSCKASGYTFTDYYVNWVRQAPGQGLEWMGVINPHNGDTRYNQKFKGRVTMTRDTSTSTVYMELSSLRSEDTAVYYCASWLRRGYYFDSWGQGTTVTVSS

SEQ ID NO: 29 - protein, 119 aa, artificial sequence
QVQLVQSGAEVKKPGASVKVSCKASGYTFTDYYVNWVRQAPGQGLEWMGVINPHNGDTRYNQKFKGRVTMTVDKSTSTVYMELSSLRSEDTAVYYCASWLRRGYYFDSWGQGTTVTVSS

SEQ ID NO: 30 - protein, 119 aa, artificial sequence
QVQLVQSGAEVKKPGASVKVSCKASGYTFTDYYVNWVRQAPGQGLEWIGVINPHNGDTRYNQKFKGRATLTVDKSTSTVYMELSSLRSEDTAVYYCASWLRRGYYFDSWGQGTTVTVSS

SEQ ID NO: 31 - protein, 119 aa, artificial sequence
KVQLVQSGAEVKKPGASVKVSCKASGYTFTDYYVNWVRQAPGQGLEWIGVINPHNGDTRYNQKFKGKATLTVDKSTSTAYMELSSLRSEDTAVYYCASWLRRGYYFDSWGQGTTVTVSS

SEQ ID NO: 32 - protein, 127 aa, artificial sequence
QVQLVQSGAEVKKPGSSVKVSCKASGGTFSGYNMNWVRQAPGQGLEWMGNIDPYYGGTNYNQKFKGRVTITADKSTSTAYMELSSLRSEDTAVYYCARETWFITTGVIKKGFYFDYWGQGTTVTVSS

SEQ ID NO: 33 - protein, 127 aa, artificial sequence
QVQLVQSGAEVKKPGSSVKVSCKASGYSFTGYNMNWVRQAPGQGLEWMGNIDPYYGGTNYNQKFKGRVTITADKSTSTAYMELSSLRSEDTAVYYCARETWFITTGVIKKGFYFDYWGQGTTVTVSS

SEQ ID NO: 34 - protein, 127 aa, artificial sequence
QVQLVQSGAEVKKPGSSVKVSCKASGGTFSGYNMNWVRQAPGQGLEWMGNIDPYYGGTNYNQKFKGKATITADKSTSTAYMELSSLRSEDTAVYYCARETWFITTGVIKKGFYFDYWGQGTTVTVSS

SEQ ID NO: 35 - protein, 127 aa, artificial sequence
QVQLVQSGAEVKKPGSSVKVSCKASGYSFTGYNMNWVRQAPGQGLEWMGNIDPYYGGTNYNQKFKGKATITADKSTSTAYMELSSLRSEDTAVYYCARETWFITTGVIKKGFYFDYWGQGTTVTVSS

SEQ ID NO: 36 - protein, 123 aa, artificial sequence
EVQLIESGGGLVQPKGSLKLSCAASGFNFNAYAMNWVRQAPGKGLEWVARIRSKSNNFATYYADSVTDRFTISRDDSESMLYLQMNNLKTEDTAMYYCVRHGRRDLLYSMDFWGQGTSVTVSS

SEQ ID NO: 37 - protein, 123 aa, artificial sequence
EVQLIESGGGLVQPKGSLKLSCAASGFNFNAYAMNWVRQAPGKGLEWVARIRSKSNDFATYYADSVKGRFTISRDDSENMLFLQMNNLKTEDTAMYYCVRHGRRDLLYSMDFWGQGTSVTVSS

SEQ ID NO: 38 - protein, 123 aa, artificial sequence
EVQLVESGGGLVQPKGSLKLSCAASGFNFNAYAMNWVRQAPGKGLEWVARIRSKSNNFATYYADSVKDRFTISRDDSESMVYLEMNNLKTEDTAMYYCVRHGRRDLLYSMDFWGQGTSVTVSS

SEQ ID NO: 39 - protein, 119 aa, artificial sequence
KVQLQQSGPVLVKPGASVKMSCKASGYTFTDYYVNWMKQNYGKSPEWIGVINPHNGDTRYNQKFKGKATLTVDKSSSTANMELTSLTSGDSAVYYCASWLRRGYYFDSWGQGTTLTVSS

SEQ ID NO: 40 - protein, 127 aa, artificial sequence
EIQLQQSGPELEKPGASVKISCKASGYSFTGYNMNWVKKSNGKSLEWIGNIDPYYGGTNYNQKFKGKATLTVDKSSSTAYMQLKSLTSEDSAVYYCARETWFITTGVIKKGFYFDYWGQGTTLTVSS

SEQ ID NO: 41 - protein, 18 aa, artificial sequence
IRSKSNDFATYYADSVKD

SEQ ID NO: 42 - protein, 112 aa, artificial sequence
DIVMTQSPLSLPVTPGEPASISCRSSKSLLHSNGITYLFWYLQKPGQSPQLLIYQMSNLASGVPDRFSGSGSGTDFTLKISRVEAEDVGVYYCAQSLELPLTFGGGTKVEIK

SEQ ID NO: 43 - protein, 112 aa, artificial sequence
DVVMTQSPLSLPVTPGEPASISCRSSKSLLHSNGITYLFWYLQKPGQSPQLLIYQMSNLASGVPDRFSGSGSGTDFTLKISRVEAEDVGVYYCAQSLELPLTFGGGTKVEIK

SEQ ID NO: 44 - protein, 107 aa, artificial sequence
EIVLTQSPATLSLSPGERATLSCRASQSISDYLHWYQQKPGQAPRLLIYYVSQSISGIPARFSGSGSGTDFTLTISSLEPEDFAVYYCQNGHSFPLTFGGGTKVEIK

SEQ ID NO: 45 - protein, 107 aa, artificial sequence
EIVLTQSPATLSLSPGERATLSCRASQSISDYLHWYQQKPGQAPRLLLKYVSQSISGIPARFSGSGSGTDFTLTISSLEPEDFAVYYCQNGHSFPLTFGGGTKVEIK

SEQ ID NO: 46 - protein, 107 aa, artificial sequence
DIVMTQSPATLSLSPGERATLSCRASQSISDYLHWYQQKPGQAPRLLLKYVSQSISGIPARFSGSGSGTDFTLTISSLEPEDFAVYYCQNGHSFPLTFGGGTKVEIK

SEQ ID NO: 47 - protein, 108 aa, artificial sequence
EIVLTQSPATLSLSPGERATLSCSASSIISSNYLHWYQQKPGQAPRLLIYRTSSLASGIPARFSGSGSGTDFTLTISSLEPEDFAVYYCQQGSSIPRTFGGGTKVEIK

SEQ ID NO: 48 - protein, 108 aa, artificial sequence
EIVLTQSPATLSLSPGERATLACSASSIISSNYLHWYQQKPGQAPRLLIYRTSSLASGIPARFSGSGSGTDYTLTISSLEPEDFAVYYCQQGSSIPRTFGGGTKVEIK

SEQ ID NO: 49 - protein, 108 aa, artificial sequence
EIVLTQSPATLSLSPGERATLACSASSIISSNYLHWYQQKPGQSPRLLIYRTSSLASGVPARFSGSGSGTSYTLTISSLEPEDFAVYYCQQGSSIPRTFGGGTKVEIK

SEQ ID NO: 50 - protein, 112 aa, artificial sequence
DVVMTQAAFSNPVTLGTSTSISCRSSKSLLHSNGITYLFWYLQKPGQSPQLLIYQMSNLASGVPDRFSGSGSGTDFTLRISRVEAEDVGVYYCAQSLELPLTFGGGTKLEIK

SEQ ID NO: 51 - protein, 112 aa, artificial sequence
DIVMTQAAFSNPVTLGTSASISCRSSKSLLHSNGITYLFWYLQKPGQSPQLLIYQMSNLASGVPDRFSGSGSGTDFTLRISRVEAEDVGVYYCAQSLELPLTFGGGTKLEIK

SEQ ID NO: 52 - protein, 112 aa, artificial sequence
DIVMTQAAFSNPVTLGTSASISCRSSKSLLHSNGITYLFWYLQKPGQSPQLLIYQMSNLASGVPDRFSGSGSGTDFTLRISRVEAEDVAVYYCAQSLELPLTFGGGTKLEIK

SEQ ID NO: 53 - protein, 107 aa, artificial sequence
DIVMTQSPATLSVTPGDRVSLSCRASQSISDYLHWYQQKSHESPRLLLKYVSQSISGIPSRFSGSGSGSDFTLTINSVEPEDVGVYYCQNGHSFPLTFGAGTKLELK

SEQ ID NO: 54 - protein, 108 aa, artificial sequence
EIVLTQSPTTMAASPGEKITLACSASSIISSNYLHWYQQKPGFSPKLLIYRTSSLASGVPARFSGSGSGTSYSLTIGTMEAEDVATYYCQQGSSIPRTFGGGTKLEIK

SEQ ID NO: 55 - protein, 453 aa, artificial sequence
EVQLVESGGGLVQPGGSLKLSCAASGFNFNAYAMNWVRQASGKGLEWVGRIRSKSNNFATYYADSVTDRFTISRDDSKNTAYLQMNSLKTEDTAVYYCVRHGRRDLLYSMDFWGQGTTVTVSSASTKGPSVFPLAPSSKSTSGGTAALGCLVKDYFPEPVTVSWNSGALTSGVHTFPAVLQSSGLYSLSSVVTVPSSSLGTQTYICNVNHKPSNTKVDKKVEPKSCDKTHTCPPCPAPELLGGPSVFLFPPKPKDTLMISRTPEVTCVVVDVSHEDPEVKFNWYVDGVEVHNAKTKPREEQYNSTYRVVSVLTVLHQDWLNGKEYKCKVSNKALPAPIEKTISKAKGQPREPQVYTLPPSRDELTKNQVSLTCLVKGFYPSDIAVEWESNGQPENNYKTTPPVLDSDGSFFLYSKLTVDKSRWQQGNVFSCSVMHEALHNHYTQKSLSLSPGK

SEQ ID NO: 56 - protein, 453 aa, artificial sequence
EVQLVESGGGLVQPGGSLKLSCAASGFTFSAYAMNWVRQASGKGLEWVGRIRSKSNNFATYYADSVTDRFTISRDDSKNTAYLQMNSLKTEDTAVYYCVRHGRRDLLYSMDFWGQGTTVTVSSASTKGPSVFPLAPSSKSTSGGTAALGCLVKDYFPEPVTVSWNSGALTSGVHTFPAVLQSSGLYSLSSVVTVPSSSLGTQTYICNVNHKPSNTKVDKKVEPKSCDKTHTCPPCPAPELLGGPSVFLFPPKPKDTLMISRTPEVTCVVVDVSHEDPEVKFNWYVDGVEVHNAKTKPREEQYNSTYRVVSVLTVLHQDWLNGKEYKCKVSNKALPAPIEKTISKAKGQPREPQVYTLPPSRDELTKNQVSLTCLVKGFYPSDIAVEWESNGQPENNYKTTPPVLDSDGSFFLYSKLTVDKSRWQQGNVFSCSVMHEALHNHYTQKSLSLSPGK

SEQ ID NO: 57 - protein, 453 aa, artificial sequence
EVQLVESGGGLVQPGGSLKLSCAASGFTFSAYAMNWVRQASGKGLEWVARIRSKSNNFATYYADSVTDRFTISRDDSKSTLYLQMNSLKTEDTAVYYCVRHGRRDLLYSMDFWGQGTTVTVSSASTKGPSVFPLAPSSKSTSGGTAALGCLVKDYFPEPVTVSWNSGALTSGVHTFPAVLQSSGLYSLSSVVTVPSSSLGTQTYICNVNHKPSNTKVDKKVEPKSCDKTHTCPPCPAPELLGGPSVFLFPPKPKDTLMISRTPEVTCVVVDVSHEDPEVKFNWYVDGVEVHNAKTKPREEQYNSTYRVVSVLTVLHQDWLNGKEYKCKVSNKALPAPIEKTISKAKGQPREPQVYTLPPSRDELTKNQVSLTCLVKGFYPSDIAVEWESNGQPENNYKTTPPVLDSDGSFFLYSKLTVDKSRWQQGNVFSCSVMHEALHNHYTQKSLSLSPGK

SEQ ID NO: 58 - protein, 453 aa, artificial sequence
EVQLVESGGGLVQPGGSLKLSCAASGFNFNAYAMNWVRQASGKGLEWVARIRSKSNNFATYYADSVTDRFTISRDDSKSTLYLQMNSLKTEDTAVYYCVRHGRRDLLYSMDFWGQGTTVTVSSASTKGPSVFPLAPSSKSTSGGTAALGCLVKDYFPEPVTVSWNSGALTSGVHTFPAVLQSSGLYSLSSVVTVPSSSLGTQTYICNVNHKPSNTKVDKKVEPKSCDKTHTCPPCPAPELLGGPSVFLFPPKPKDTLMISRTPEVTCVVVDVSHEDPEVKFNWYVDGVEVHNAKTKPREEQYNSTYRVVSVLTVLHQDWLNGKEYKCKVSNKALPAPIEKTISKAKGQPREPQVYTLPPSRDELTKNQVSLTCLVKGFYPSDIAVEWESNGQPENNYKTTPPVLDSDGSFFLYSKLTVDKSRWQQGNVFSCSVMHEALHNHYTQKSLSLSPGK

SEQ ID NO: 59 - protein, 453 aa, artificial sequence
EVQLVESGGGLVQPGGSLKLSCAASGFNFNAYAMNWVRQASGKGLEWVARIRSKSNDFATYYADSVKDRFTISRDDSKSTLYLQMNSLKTEDTAVYYCVRHGRRDLLYSMDFWGQGTTVTVSSASTKGPSVFPLAPSSKSTSGGTAALGCLVKDYFPEPVTVSWNSGALTSGVHTFPAVLQSSGLYSLSSVVTVPSSSLGTQTYICNVNHKPSNTKVDKKVEPKSCDKTHTCPPCPAPELLGGPSVFLFPPKPKDTLMISRTPEVTCVVVDVSHEDPEVKFNWYVDGVEVHNAKTKPREEQYNSTYRVVSVLTVLHQDWLNGKEYKCKVSNKALPAPIEKTISKAKGQPREPQVYTLPPSRDELTKNQVSLTCLVKGFYPSDIAVEWESNGQPENNYKTTPPVLDSDGSFFLYSKLTVDKSRWQQGNVFSCSVMHEALHNHYTQKSLSLSPGK

SEQ ID NO: 60 - protein, 453 aa, artificial sequence
EVQLVESGGGLVQPGGSLKLSCAASGFNFNAYAMNWVRQASGKGLEWVARIRSKSNDFATYYADSVKGRFTISRDDSKNTLYLQMNSLKTEDTAVYYCVRHGRRDLLYSMDFWGQGTTVTVSSASTKGPSVFPLAPSSKSTSGGTAALGCLVKDYFPEPVTVSWNSGALTSGVHTFPAVLQSSGLYSLSSVVTVPSSSLGTQTYICNVNHKPSNTKVDKKVEPKSCDKTHTCPPCPAPELLGGPSVFLFPPKPKDTLMISRTPEVTCVVVDVSHEDPEVKFNWYVDGVEVHNAKTKPREEQYNSTYRVVSVLTVLHQDWLNGKEYKCKVSNKALPAPIEKTISKAKGQPREPQVYTLPPSRDELTKNQVSLTCLVKGFYPSDIAVEWESNGQPENNYKTTPPVLDSDGSFFLYSKLTVDKSRWQQGNVFSCSVMHEALHNHYTQKSLSLSPGK

SEQ ID NO: 61 - protein, 453 aa, artificial sequence
EVQLVESGGGLVQPGGSLKLSCAASGFNFNAYAMNWVRQASGKGLEWVARIRSKSNNFATYYADSVKDRFTISRDDSKSTVYLQMNSLKTEDTAVYYCVRHGRRDLLYSMDFWGQGTTVTVSSASTKGPSVFPLAPSSKSTSGGTAALGCLVKDYFPEPVTVSWNSGALTSGVHTFPAVLQSSGLYSLSSVVTVPSSSLGTQTYICNVNHKPSNTKVDKKVEPKSCDKTHTCPPCPAPELLGGPSVFLFPPKPKDTLMISRTPEVTCVVVDVSHEDPEVKFNWYVDGVEVHNAKTKPREEQYNSTYRVVSVLTVLHQDWLNGKEYKCKVSNKALPAPIEKTISKAKGQPREPQVYTLPPSRDELTKNQVSLTCLVKGFYPSDIAVEWESNGQPENNYKTTPPVLDSDGSFFLYSKLTVDKSRWQQGNVFSCSVMHEALHNHYTQKSLSLSPGK

SEQ ID NO: 62 - protein, 453 aa, artificial sequence
EVQLVESGGGLVQPGGSLKLSCAASGFNFNAYAMNWVRQASGKGLEWVGRIRSKSNNFATYYADSVTDRFTISRDDSKNTAYLQMNSLKTEDTAVYYCVRHGRRDLLYSMDFWGQGTTVTVSSASTKGPSVFPLAPSSKSTSGGTAALGCLVKDYFPEPVTVSWNSGALTSGVHTFPAVLQSSGLYSLSSVVTVPSSSLGTQTYICNVNHKPSNTKVDKKVEPKSCDKTHTCPPCPAPELVGGPSVFLLPPKPKDTLMISRTPEVTCVVVDVSHEDPEVKFNWYVDGVEVHNAKTKPPEEQYNSTLRVVSVLTVLHQDWLNGKEYKCKVSNKALPAPIEKTISKAKGQPREPQVYTLPPSRDELTKNQVSLTCLVKGFYPSDIAVEWESNGQPENNYKTTPLVLDSDGSFFLYSKLTVDKSRWQQGNVFSCSVMHEALHNHYTQKSLSLSPGK

SEQ ID NO: 63 - protein, 453 aa, artificial sequence
EVQLVESGGGLVQPGGSLKLSCAASGFNFNAYAMNWVRQASGKGLEWVGRIRSKSNNFATYYADSVTDRFTISRDDSKNTAYLQMNSLKTEDTAVYYCVRHGRRDLLYSMDFWGQGTTVTVSSASTKGPSVFPLAPSSKSTSGGTAALGCLVKDYFPEPVTVSWNSGALTSGVHTFPAVLQSSGLYSLSSVVTVPSSSLGTQTYICNVNHKPSNTKVDKKVEPKSCDKTHTCPPCPAPELLGGPDVFLFPPKPKDTLMISRTPEVTCVVVDVSHEDPEVKFNWYVDGVEVHNAKTKPREEQYNSTYRVVSVLTVLHQDWLNGKEYKCKVSNKALPAPEEKTISKAKGQPREPQVYTLPPSRDELTKNQVSLTCLVKGFYPSDIAVEWESNGQPENNYKTTPPVLDSDGSFFLYSKLTVDKSRWQQGNVFSCSVMHEALHNHYTQKSLSLSPGK

SEQ ID NO: 64 - protein, 453 aa, artificial sequence
EVQLVESGGGLVQPGGSLKLSCAASGFNFNAYAMNWVRQASGKGLEWVGRIRSKSNNFATYYADSVTDRFTISRDDSKNTAYLQMNSLKTEDTAVYYCVRHGRRDLLYSMDFWGQGTTVTVSSASTKGPSVFPLAPSSKSTSGGTAALGCLVKDYFPEPVTVSWNSGALTSGVHTFPAVLQSSGLYSLSSVVTVPSSSLGTQTYICNVNHKPSNTKVDKKVEPKSCDKTHTCPPCPAPELLGGPDVFLFPPKPKDTLMISRTPEVTCVVVDVSHEDPEVKFNWYVDGVEVHNAKTKPREEQYNSTYRVVSVLTVLHQDWLNGKEYKCKVSNKALPLPEEKTISKAKGQPREPQVYTLPPSRDELTKNQVSLTCLVKGFYPSDIAVEWESNGQPENNYKTTPPVLDSDGSFFLYSKLTVDKSRWQQGNVFSCSVMHEALHNHYTQKSLSLSPGK

SEQ ID NO: 65 - protein, 449 aa, artificial sequence
QVQLVQSGAEVKKPGASVKVSCKASGYTFTDYYVNWVRQAPGQGLEWMGVINPHNGDTRYNQKFKGRVTMTRDTSTSTVYMELSSLRSEDTAVYYCASWLRRGYYFDSWGQGTTVTVSSASTKGPSVFPLAPSSKSTSGGTAALGCLVKDYFPEPVTVSWNSGALTSGVHTFPAVLQSSGLYSLSSVVTVPSSSLGTQTYICNVNHKPSNTKVDKKVEPKSCDKTHTCPPCPAPELLGGPSVFLFPPKPKDTLMISRTPEVTCVVVDVSHEDPEVKFNWYVDGVEVHNAKTKPREEQYNSTYRVVSVLTVLHQDWLNGKEYKCKVSNKALPAPIEKTISKAKGQPREPQVYTLPPSRDELTKNQVSLTCLVKGFYPSDIAVEWESNGQPENNYKTTPPVLDSDGSFFLYSKLTVDKSRWQQGNVFSCSVMHEALHNHYTQKSLSLSPGK

SEQ ID NO: 66 - protein, 449 aa, artificial sequence
QVQLVQSGAEVKKPGASVKVSCKASGYTFTDYYVNWVRQAPGQGLEWMGVINPHNGDTRYNQKFKGRVTMTVDKSTSTVYMELSSLRSEDTAVYYCASWLRRGYYFDSWGQGTTVTVSSASTKGPSVFPLAPSSKSTSGGTAALGCLVKDYFPEPVTVSWNSGALTSGVHTFPAVLQSSGLYSLSSVVTVPSSSLGTQTYICNVNHKPSNTKVDKKVEPKSCDKTHTCPPCPAPELLGGPSVFLFPPKPKDTLMISRTPEVTCVVVDVSHEDPEVKFNWYVDGVEVHNAKTKPREEQYNSTYRVVSVLTVLHQDWLNGKEYKCKVSNKALPAPIEKTISKAKGQPREPQVYTLPPSRDELTKNQVSLTCLVKGFYPSDIAVEWESNGQPENNYKTTPPVLDSDGSFFLYSKLTVDKSRWQQGNVFSCSVMHEALHNHYTQKSLSLSPGK

SEQ ID NO: 67 - protein, 449 aa, artificial sequence
QVQLVQSGAEVKKPGASVKVSCKASGYTFTDYYVNWVRQAPGQGLEWIGVINPHNGDTRYNQKFKGRATLTVDKSTSTVYMELSSLRSEDTAVYYCASWLRRGYYFDSWGQGTTVTVSSASTKGPSVFPLAPSSKSTSGGTAALGCLVKDYFPEPVTVSWNSGALTSGVHTFPAVLQSSGLYSLSSVVTVPSSSLGTQTYICNVNHKPSNTKVDKKVEPKSCDKTHTCPPCPAPELLGGPSVFLFPPKPKDTLMISRTPEVTCVVVDVSHEDPEVKFNWYVDGVEVHNAKTKPREEQYNSTYRVVSVLTVLHQDWLNGKEYKCKVSNKALPAPIEKTISKAKGQPREPQVYTLPPSRDELTKNQVSLTCLVKGFYPSDIAVEWESNGQPENNYKTTPPVLDSDGSFFLYSKLTVDKSRWQQGNVFSCSVMHEALHNHYTQKSLSLSPGK

SEQ ID NO: 68 - protein, 449 aa, artificial sequence
KVQLVQSGAEVKKPGASVKVSCKASGYTFTDYYVNWVRQAPGQGLEWIGVINPHNGDTRYNQKFKGKATLTVDKSTSTAYMELSSLRSEDTAVYYCASWLRRGYYFDSWGQGTTVTVSSASTKGPSVFPLAPSSKSTSGGTAALGCLVKDYFPEPVTVSWNSGALTSGVHTFPAVLQSSGLYSLSSVVTVPSSSLGTQTYICNVNHKPSNTKVDKKVEPKSCDKTHTCPPCPAPELLGGPSVFLFPPKPKDTLMISRTPEVTCVVVDVSHEDPEVKFNWYVDGVEVHNAKTKPREEQYNSTYRVVSVLTVLHQDWLNGKEYKCKVSNKALPAPIEKTISKAKGQPREPQVYTLPPSRDELTKNQVSLTCLVKGFYPSDIAVEWESNGQPENNYKTTPPVLDSDGSFFLYSKLTVDKSRWQQGNVFSCSVMHEALHNHYTQKSLSLSPGK

SEQ ID NO: 69 - protein, 449 aa, artificial sequence
QVQLVQSGAEVKKPGASVKVSCKASGYTFTDYYVNWVRQAPGQGLEWMGVINPHNGDTRYNQKFKGRVTMTVDKSTSTVYMELSSLRSEDTAVYYCASWLRRGYYFDSWGQGTTVTVSSASTKGPSVFPLAPSSKSTSGGTAALGCLVKDYFPEPVTVSWNSGALTSGVHTFPAVLQSSGLYSLSSVVTVPSSSLGTQTYICNVNHKPSNTKVDKKVEPKSCDKTHTCPPCPAPELLGGPDVFLFPPKPKDTLMISRTPEVTCVVVDVSHEDPEVKFNWYVDGVEVHNAKTKPREEQYNSTYRVVSVLTVLHQDWLNGKEYKCKVSNKALPAPEEKTISKAKGQPREPQVYTLPPSRDELTKNQVSLTCLVKGFYPSDIAVEWESNGQPENNYKTTPPVLDSDGSFFLYSKLTVDKSRWQQGNVFSCSVMHEALHNHYTQKSLSLSPGK

SEQ ID NO: 70 - protein, 449 aa, artificial sequence
QVQLVQSGAEVKKPGASVKVSCKASGYTFTDYYVNWVRQAPGQGLEWMGVINPHNGDTRYNQKFKGRVTMTVDKSTSTVYMELSSLRSEDTAVYYCASWLRRGYYFDSWGQGTTVTVSSASTKGPSVFPLAPSSKSTSGGTAALGCLVKDYFPEPVTVSWNSGALTSGVHTFPAVLQSSGLYSLSSVVTVPSSSLGTQTYICNVNHKPSNTKVDKKVEPKSCDKTHTCPPCPAPELVGGPSVFLLPPKPKDTLMISRTPEVTCVVVDVSHEDPEVKFNWYVDGVEVHNAKTKPPEEQYNSTLRVVSVLTVLHQDWLNGKEYKCKVSNKALPAPIEKTISKAKGQPREPQVYTLPPSRDELTKNQVSLTCLVKGFYPSDIAVEWESNGQPENNYKTTPLVLDSDGSFFLYSKLTVDKSRWQQGNVFSCSVMHEALHNHYTQKSLSLSPGK

SEQ ID NO: 71 - protein, 457 aa, artificial sequence
QVQLVQSGAEVKKPGSSVKVSCKASGGTFSGYNMNWVRQAPGQGLEWMGNIDPYYGGTNYNQKFKGRVTITADKSTSTAYMELSSLRSEDTAVYYCARETWFITTGVIKKGFYFDYWGQGTTVTVSSASTKGPSVFPLAPSSKSTSGGTAALGCLVKDYFPEPVTVSWNSGALTSGVHTFPAVLQSSGLYSLSSVVTVPSSSLGTQTYICNVNHKPSNTKVDKKVEPKSCDKTHTCPPCPAPELLGGPSVFLFPPKPKDTLMISRTPEVTCVVVDVSHEDPEVKFNWYVDGVEVHNAKTKPREEQYNSTYRVVSVLTVLHQDWLNGKEYKCKVSNKALPAPIEKTISKAKGQPREPQVYTLPPSRDELTKNQVSLTCLVKGFYPSDIAVEWESNGQPENNYKTTPPVLDSDGSFFLYSKLTVDKSRWQQGNVFSCSVMHEALHNHYTQKSLSLSPGK

SEQ ID NO: 72 - protein, 457 aa, artificial sequence
QVQLVQSGAEVKKPGSSVKVSCKASGYSFTGYNMNWVRQAPGQGLEWMGNIDPYYGGTNYNQKFKGRVTITADKSTSTAYMELSSLRSEDTAVYYCARETWFITTGVIKKGFYFDYWGQGTTVTVSSASTKGPSVFPLAPSSKSTSGGTAALGCLVKDYFPEPVTVSWNSGALTSGVHTFPAVLQSSGLYSLSSVVTVPSSSLGTQTYICNVNHKPSNTKVDKKVEPKSCDKTHTCPPCPAPELLGGPSVFLFPPKPKDTLMISRTPEVTCVVVDVSHEDPEVKFNWYVDGVEVHNAKTKPREEQYNSTYRVVSVLTVLHQDWLNGKEYKCKVSNKALPAPIEKTISKAKGQPREPQVYTLPPSRDELTKNQVSLTCLVKGFYPSDIAVEWESNGQPENNYKTTPPVLDSDGSFFLYSKLTVDKSRWQQGNVFSCSVMHEALHNHYTQKSLSLSPGK

SEQ ID NO: 73 - protein, 457 aa, artificial sequence
QVQLVQSGAEVKKPGSSVKVSCKASGGTFSGYNMNWVRQAPGQGLEWMGNIDPYYGGTNYNQKFKGKATITADKSTSTAYMELSSLRSEDTAVYYCARETWFITTGVIKKGFYFDYWGQGTTVTVSSASTKGPSVFPLAPSSKSTSGGTAALGCLVKDYFPEPVTVSWNSGALTSGVHTFPAVLQSSGLYSLSSVVTVPSSSLGTQTYICNVNHKPSNTKVDKKVEPKSCDKTHTCPPCPAPELLGGPSVFLFPPKPKDTLMISRTPEVTCVVVDVSHEDPEVKFNWYVDGVEVHNAKTKPREEQYNSTYRVVSVLTVLHQDWLNGKEYKCKVSNKALPAPIEKTISKAKGQPREPQVYTLPPSRDELTKNQVSLTCLVKGFYPSDIAVEWESNGQPENNYKTTPPVLDSDGSFFLYSKLTVDKSRWQQGNVFSCSVMHEALHNHYTQKSLSLSPGK

SEQ ID NO: 74 - protein, 457 aa, artificial sequence
QVQLVQSGAEVKKPGSSVKVSCKASGYSFTGYNMNWVRQAPGQGLEWMGNIDPYYGGTNYNQKFKGKATITADKSTSTAYMELSSLRSEDTAVYYCARETWFITTGVIKKGFYFDYWGQGTTVTVSSASTKGPSVFPLAPSSKSTSGGTAALGCLVKDYFPEPVTVSWNSGALTSGVHTFPAVLQSSGLYSLSSVVTVPSSSLGTQTYICNVNHKPSNTKVDKKVEPKSCDKTHTCPPCPAPELLGGPSVFLFPPKPKDTLMISRTPEVTCVVVDVSHEDPEVKFNWYVDGVEVHNAKTKPREEQYNSTYRVVSVLTVLHQDWLNGKEYKCKVSNKALPAPIEKTISKAKGQPREPQVYTLPPSRDELTKNQVSLTCLVKGFYPSDIAVEWESNGQPENNYKTTPPVLDSDGSFFLYSKLTVDKSRWQQGNVFSCSVMHEALHNHYTQKSLSLSPGK

SEQ ID NO: 75 - protein, 219 aa, artificial sequence
DIVMTQSPLSLPVTPGEPASISCRSSKSLLHSNGITYLFWYLQKPGQSPQLLIYQMSNLASGVPDRFSGSGSGTDFTLKISRVEAEDVGVYYCAQSLELPLTFGGGTKVEIKRTVAAPSVFIFPPSDEQLKSGTASVVCLLNNFYPREAKVQWKVDNALQSGNSQESVTEQDSKDSTYSLSSTLTLSKADYEKHKVYACEVTHQGLSSPVTKSFNRGEC

SEQ ID NO: 76 - protein, 219 aa, artificial sequence
DVVMTQSPLSLPVTPGEPASISCRSSKSLLHSNGITYLFWYLQKPGQSPQLLIYQMSNLASGVPDRFSGSGSGTDFTLKISRVEAEDVGVYYCAQSLELPLTFGGGTKVEIKRTVAAPSVFIFPPSDEQLKSGTASVVCLLNNFYPREAKVQWKVDNALQSGNSQESVTEQDSKDSTYSLSSTLTLSKADYEKHKVYACEVTHQGLSSPVTKSFNRGEC

SEQ ID NO: 77 - protein, 214 aa, artificial sequence
EIVLTQSPATLSLSPGERATLSCRASQSISDYLHWYQQKPGQAPRLLIYYVSQSISGIPARFSGSGSGTDFTLTISSLEPEDFAVYYCQNGHSFPLTFGGGTKVEIKRTVAAPSVFIFPPSDEQLKSGTASVVCLLNNFYPREAKVQWKVDNALQSGNSQESVTEQDSKDSTYSLSSTLTLSKADYEKHKVYACEVTHQGLSSPVTKSFNRGEC

SEQ ID NO: 78 - protein, 214 aa, artificial sequence
EIVLTQSPATLSLSPGERATLSCRASQSISDYLHWYQQKPGQAPRLLLKYVSQSISGIPARFSGSGSGTDFTLTISSLEPEDFAVYYCQNGHSFPLTFGGGTKVEIKRTVAAPSVFIFPPSDEQLKSGTASVVCLLNNFYPREAKVQWKVDNALQSGNSQESVTEQDSKDSTYSLSSTLTLSKADYEKHKVYACEVTHQGLSSPVTKSFNRGEC

SEQ ID NO: 79 - protein, 214 aa, artificial sequence
DIVMTQSPATLSLSPGERATLSCRASQSISDYLHWYQQKPGQAPRLLLKYVSQSISGIPARFSGSGSGTDFTLTISSLEPEDFAVYYCQNGHSFPLTFGGGTKVEIKRTVAAPSVFIFPPSDEQLKSGTASVVCLLNNFYPREAKVQWKVDNALQSGNSQESVTEQDSKDSTYSLSSTLTLSKADYEKHKVYACEVTHQGLSSPVTKSFNRGEC

SEQ ID NO: 80 - protein, 215 aa, artificial sequence
EIVLTQSPATLSLSPGERATLSCSASSIISSNYLHWYQQKPGQAPRLLIYRTSSLASGIPARFSGSGSGTDFTLTISSLEPEDFAVYYCQQGSSIPRTFGGGTKVEIKRTVAAPSVFIFPPSDEQLKSGTASVVCLLNNFYPREAKVQWKVDNALQSGNSQESVTEQDSKDSTYSLSSTLTLSKADYEKHKVYACEVTHQGLSSPVTKSFNRGEC

SEQ ID NO: 81 - protein, 215 aa, artificial sequence
EIVLTQSPATLSLSPGERATLACSASSIISSNYLHWYQQKPGQAPRLLIYRTSSLASGIPARFSGSGSGTDYTLTISSLEPEDFAVYYCQQGSSIPRTFGGGTKVEIKRTVAAPSVFIFPPSDEQLKSGTASVVCLLNNFYPREAKVQWKVDNALQSGNSQESVTEQDSKDSTYSLSSTLTLSKADYEKHKVYACEVTHQGLSSPVTKSFNRGEC

SEQ ID NO: 82 - protein, 215 aa, artificial sequence
EIVLTQSPATLSLSPGERATLACSASSIISSNYLHWYQQKPGQSPRLLIYRTSSLASGVPARFSGSGSGTSYTLTISSLEPEDFAVYYCQQGSSIPRTFGGGTKVEIKRTVAAPSVFIFPPSDEQLKSGTASVVCLLNNFYPREAKVQWKVDNALQSGNSQESVTEQDSKDSTYSLSSTLTLSKADYEKHKVYACEVTHQGLSSPVTKSFNRGEC

SEQ ID NO: 83 - protein, 330 aa, artificial sequence
AKTTAPSVYPLAPVCGDTTGSSVTLGCLVKGYFPEPVTLTWNSGSLSSGVHTFPAVLQSDLYTLSSSVTVTSSTWPSQSITCNVAHPASSTKVDKKIEPRGPTIKPCPPCKCPAPNLLGGPSVFIFPPKIKDVLMISLSPIVTCVVVDVSEDDPDVQISWFVNNVEVHTAQTQTHREDYNSTLRVVSALPIQHQDWMSGKEFKCKVNNKDLPAPIERTISKPKGSVRAPQVYVLPPPEEEMTKKQVTLTCMVTDFMPEDIYVEWTNNGKTELNYKNTEPVLDSDGSYFMYSKLRVEKKNWVERNSYSCSVVHEGLHNHHTTKSFSRTPGK

SEQ ID NO: 84 - protein, 107 aa, artificial sequence
RADAAPTVSIFPPSSEQLTSGGASVVCFLNNFYPKDINVKWKIDGSERQNGVLNSWTDQDSKDSTYSMSSTLTLTKDEYERHNSYTCEATHKTSTSPIVKSFNRNEC

SEQ ID NO: 85 - protein, 330 aa, artificial sequence [sequence omitted]

SEQ ID NO: 86 - protein, 107 aa, artificial sequence [sequence omitted]

SEQ ID NO: 87 - protein, 330 aa, artificial sequence
ASTKGPSVFPLAPSSKSTSGGTAALGCLVKDYFPEPVTVSWNSGALTSGVHTFPAVLQSSGLYSLSSVVTVPSSSLGTQTYICNVNHKPSNTKVDKKVEPKSCDKTHTCPPCPAPELVGGPSVFLLPPKPKDTLMISRTPEVTCVVVDVSHEDPEVKFNWYVDGVEVHNAKTKPPEEQYNSTLRVVSVLTVLHQDWLNGKEYKCKVSNKALPAPIEKTISKAKGQPREPQVYTLPPSRDELTKNQVSLTCLVKGFYPSDIAVEWESNGQPENNYKTTPLVLDSDGSFFLYSKLTVDKSRWQQGNVFSCSVMHEALHNHYTQKSLSLSPGK

SEQ ID NO: 88 - protein, 330 aa, artificial sequence
ASTKGPSVFPLAPSSKSTSGGTAALGCLVKDYFPEPVTVSWNSGALTSGVHTFPAVLQSSGLYSLSSVVTVPSSSLGTQTYICNVNHKPSNTKVDKKVEPKSCDKTHTCPPCPAPELLGGPDVFLFPPKPKDTLMISRTPEVTCVVVDVSHEDPEVKFNWYVDGVEVHNAKTKPREEQYNSTYRVVSVLTVLHQDWLNGKEYKCKVSNKALPAPEEKTISKAKGQPREPQVYTLPPSRDELTKNQVSLTCLVKGFYPSDIAVEWESNGQPENNYKTTPPVLDSDGSFFLYSKLTVDKSRWQQGNVFSCSVMHEALHNHYTQKSLSLSPGK

SEQ ID NO: 89 - protein, 330 aa, artificial sequence
ASTKGPSVFPLAPSSKSTSGGTAALGCLVKDYFPEPVTVSWNSGALTSGVHTFPAVLQSSGLYSLSSVVTVPSSSLGTQTYICNVNHKPSNTKVDKKVEPKSCDKTHTCPPCPAPELLGGPDVFLFPPKPKDTLMISRTPEVTCVVVDVSHEDPEVKFNWYVDGVEVHNAKTKPREEQYNSTYRVVSVLTVLHQDWLNGKEYKCKVSNKALPLPEEKTISKAKGQPREPQVYTLPPSRDELTKNQVSLTCLVKGFYPSDIAVEWESNGQPENNYKTTPPVLDSDGSFFLYSKLTVDKSRWQQGNVFSCSVMHEALHNHYTQKSLSLSPGK

SEQ ID NO: 90 - protein, 88 aa, artificial sequence
EIVLTQSPATLSLSPGERATLSCRASQSVSSYLAWYQQKPGQAPRLLIYDASNRATGIPARFSGSGSGTDFTLTISSLEPEDFAVYYC

SEQ ID NO: 91 - protein, 98 aa, artificial sequence
QVQLVQSGAEVKKPGSSVKVSCKASGGTFSSYAISWVRQAPGQGLEWMGGIIPIFGTANYAQKFQGRVTITADKSTSTAYMELSSLRSEDTAVYYCAR

SEQ ID NO: 92 - protein, 96 aa, artificial sequence
QVQLVQSGAEVKKPGASVKVSCKASGYTFTSYYMHWVRQAPGQGLEWMGIINPSGGSTSYAQKFQGRVTMTRDTSTSTVYMELSSLRSEDTAVYYC

SEQ ID NO: 93 - protein, 88 aa, artificial sequence; identical to SEQ ID NO: 90

SEQ ID NO: 94 - protein, 98 aa, artificial sequence
EVQLVESGGGLVQPGGSLKLSCAASGFTFSGSAMHWVRQASGKGLEWVGRIRSKANSYATAYAASVKGRFTISRDDSKNTAYLQMNSLKTEDTAVYYC

SEQ ID NO: 95 - protein, 93 aa, artificial sequence
DIVMTQSPLSLPVTPGEPASISCRSSQSLLHSNGYNYLDWYLQKPGQSPQLLIYLGSNRASGVPDRFSGSGSGTDFTLKISRVEAEDVGVYYC